European Patent Specification EP 3 866 786 B1, published September 18, 2024. Title: COMPOSITIONS AND METHODS FOR SUPPRESSING AND/OR TREATING METABOLIC DISEASES AND/OR A CLINICAL CONDITION THEREOF. Applicant: CK Biotechnology Co. The sequence listing filed with the application follows.

SEQUENCE LISTING (74 sequences)

SEQ ID NO: 1 - DNA, 22 bp, Artificial Sequence
  CXXC5 Forward Primer
caagaagaagcggaaacgctgc

SEQ ID NO: 2 - DNA, 22 bp, Artificial Sequence
  CXXC5 Reverse Primer
tctccagagcagcggaaggctt

SEQ ID NO: 3 - DNA, 20 bp, Artificial Sequence
  CXXC4 Forward Primer
caacccagccaagaagaaga

SEQ ID NO: 4 - DNA, 20 bp, Artificial Sequence
  CXXC4 Reverse Primer
agatctggtgtcccgttttg

SEQ ID NO: 5 - DNA, 23 bp, Artificial Sequence
  Tcf4 Forward Primer
tgtgtacccaatcacgacaggag

SEQ ID NO: 6 - DNA, 20 bp, Artificial Sequence
  Tcf4 Reverse Primer
gattccggtcgtgtgcagag

SEQ ID NO: 7 - DNA, 20 bp, Artificial Sequence
  Axin2 Forward Primer
tggagagtgagcggcagagc

SEQ ID NO: 8 - DNA, 18 bp, Artificial Sequence
  Axin2 Reverse Primer
tggagacgagcgggcaga

SEQ ID NO: 9 - DNA, 19 bp, Artificial Sequence
  Dvl1 Forward Primer
ccttccatccaaatgttgc

SEQ ID NO: 10 - DNA, 23 bp, Artificial Sequence
  Dvl1 Reverse Primer
gtgactgaccatagactctgtgc

SEQ ID NO: 11 - DNA, 22 bp, Artificial Sequence
  Wisp1 Forward Primer
atcgcccgaggtacgcaatagg

SEQ ID NO: 12 - DNA, 21 bp, Artificial Sequence
  Wisp1 Reverse Primer
cagcccaccgtgccatcaatg

SEQ ID NO: 13 - DNA, 20 bp, Artificial Sequence
  Fosl1 Forward Primer
aaccggaggaaggaactgac

SEQ ID NO: 14 - DNA, 20 bp, Artificial Sequence
  Fosl1 Reverse Primer
aaccggaggaaggaactgac

SEQ ID NO: 15 - DNA, 21 bp, Artificial Sequence
  PPARgamma Forward Primer
tgtggggataaagcatcaggc

SEQ ID NO: 16 - DNA, 23 bp, Artificial Sequence
  PPARgamma Reverse Primer
ccggcagttaagatcacacctat

SEQ ID NO: 17 - DNA, 21 bp, Artificial Sequence
  C/EBPalpha Forward Primer
ggtggacaagaacagcaacga

SEQ ID NO: 18 - DNA, 21 bp, Artificial Sequence
  C/EBPalpha Reverse Primer
tgtccagttcacggctcagct

SEQ ID NO: 19 - DNA, 20 bp, Artificial Sequence
  SREBP1 Forward Primer
ggagccatggattgcacatt

SEQ ID NO: 20 - DNA, 18 bp, Artificial Sequence
  SREBP1 Reverse Primer
ggcccgggaagtcactgt

SEQ ID NO: 21 - DNA, 21 bp, Artificial Sequence
  FAS Forward Primer
gcgatgaagagcatggtttag

SEQ ID NO: 22 - DNA, 19 bp, Artificial Sequence
  FAS Reverse Primer
ggctcaagggttccatgtt

SEQ ID NO: 23 - DNA, 22 bp, Artificial Sequence
  SCD-1 Forward Primer
ctgtacgggatcatactggttc

SEQ ID NO: 24 - DNA, 20 bp, Artificial Sequence
  SCD-1 Reverse Primer
gccgtgccttgtaagttctg

SEQ ID NO: 25 - DNA, 20 bp, Artificial Sequence
  ACC Forward Primer
cctccgtcagctcagataca

SEQ ID NO: 26 - DNA, 22 bp, Artificial Sequence
  ACC Reverse Primer
tttactaggtgcaagccagaca

SEQ ID NO: 27 - DNA, 16 bp, Artificial Sequence
  TNFalpha Forward Primer
cggagtccgggcaggt

SEQ ID NO: 28 - DNA, 20 bp, Artificial Sequence
  TNFalpha Reverse Primer
gctgggtagagaatggatca

SEQ ID NO: 29 - DNA, 22 bp, Artificial Sequence
  TGFbeta1 Forward Primer
tgacgtcactggagttgtacgg

SEQ ID NO: 30 - DNA, 21 bp, Artificial Sequence
  TGFbeta1 Reverse Primer
ggttcatgtcatggatggtgc

SEQ ID NO: 31 - DNA, 24 bp, Artificial Sequence
  IFNgamma Forward Primer
tcaagtggcatagatgtggaagaa

SEQ ID NO: 32 - DNA, 21 bp, Artificial Sequence
  IFNgamma Reverse Primer
tggctctgcaggattttcatg

SEQ ID NO: 33 - DNA, 22 bp, Artificial Sequence
  F4/80 Forward Primer
ctttggctatgggcttccagtc

SEQ ID NO: 34 - DNA, 24 bp, Artificial Sequence
  F4/80 Reverse Primer
gcaaggaggacagagtttatcgtg

SEQ ID NO: 35 - DNA, 24 bp, Artificial Sequence
  MCP1 Forward Primer
actgaagccagctctctcttcctc

SEQ ID NO: 36 - DNA, 24 bp, Artificial Sequence
  MCP1 Reverse Primer
ttccttcttggggtcagcacagac

SEQ ID NO: 37 - DNA, 22 bp, Artificial Sequence
  Arg1 Forward Primer
ctccaagccaaagtccttagag

SEQ ID NO: 38 - DNA, 22 bp, Artificial Sequence
  Arg1 Reverse Primer
ggagctgtcattagggacatca

SEQ ID NO: 39 - DNA, 22 bp, Artificial Sequence
  Chi3l3 Forward Primer
caggtctggcaattcttctgaa

SEQ ID NO: 40 - DNA, 23 bp, Artificial Sequence
  Chi3l3 Reverse Primer
gtcttgctcatgtgtgtaagtga

SEQ ID NO: 41 - DNA, 23 bp, Artificial Sequence
  Retnla Forward Primer
ccaatccagctaactatccctcc

SEQ ID NO: 42 - DNA, 20 bp, Artificial Sequence
  Retnla Reverse Primer
acccagtagcagtcatccca

SEQ ID NO: 43 - DNA, 20 bp, Artificial Sequence
  Pdcd1lg2 Forward Primer
ttgtcggtgtgattggcttc

SEQ ID NO: 44 - DNA, 20 bp, Artificial Sequence
  Pdcd1lg2 Reverse Primer
aaaaggcagcacacagttgc

SEQ ID NO: 45 - DNA, 21 bp, Artificial Sequence
  IL-10 Forward Primer
gctatgctgcctgctcttact

SEQ ID NO: 46 - DNA, 19 bp, Artificial Sequence
  IL-10 Reverse Primer
cctgctgatcctcatgcca

SEQ ID NO: 47 - DNA, 21 bp, Artificial Sequence
  Irs1 Forward Primer
ggacttgagctatgacacggg

SEQ ID NO: 48 - DNA, 23 bp, Artificial Sequence
  Irs1 Reverse Primer
gccaatcaggttctttgtctgac

SEQ ID NO: 49 - DNA, 18 bp, Artificial Sequence
  G6pc Forward Primer
gtcgtggctggagtcttg

SEQ ID NO: 50 - DNA, 18 bp, Artificial Sequence
  G6pc Reverse Primer
cggaggctggcattgtag

SEQ ID NO: 51 - DNA, 22 bp, Artificial Sequence
  PEPCK Forward Primer
atctcctttggaagcggatatg

SEQ ID NO: 52 - DNA, 20 bp, Artificial Sequence
  PEPCK Reverse Primer
cgcaacgcaaagcatttctt

SEQ ID NO: 53 - DNA, 20 bp, Artificial Sequence
  Pck1 Forward Primer
ggtattgaactgacagactc

SEQ ID NO: 54 - DNA, 18 bp, Artificial Sequence
  Pck1 Reverse Primer
ccagttgttgaccaaagg

SEQ ID NO: 55 - DNA, 23 bp, Artificial Sequence
  Fbp1 Forward Primer
gtaacatctacagccttaatgag

SEQ ID NO: 56 - DNA, 19 bp, Artificial Sequence
  Fbp1 Reverse Primer
ccagagtgcggtgaatatc

SEQ ID NO: 57 - DNA, 21 bp, Artificial Sequence
  UCP1 Forward Primer
aggcttccagtaccattaggt

SEQ ID NO: 58 - DNA, 22 bp, Artificial Sequence
  UCP1 Reverse Primer
ctgagtgaggcaaagctgattt

SEQ ID NO: 59 - DNA, 19 bp, Artificial Sequence
  SIRT1 Forward Primer
ttggcaccgatcctcgaac

SEQ ID NO: 60 - DNA, 21 bp, Artificial Sequence
  SIRT1 Reverse Primer
cccagctccagtcagaactat

SEQ ID NO: 61 - DNA, 23 bp, Artificial Sequence
  Dio2 Forward Primer
cagtgtggtgcacgtctccaatc

SEQ ID NO: 62 - DNA, 21 bp, Artificial Sequence
  Dio2 Reverse Primer
tgaaccaaagttgaccaccag

SEQ ID NO: 63 - DNA, 22 bp, Artificial Sequence
  PGC1alpha Forward Primer
agccgtgaccactgacaacgag

SEQ ID NO: 64 - DNA, 23 bp, Artificial Sequence
  PGC1alpha Reverse Primer
gctgcatggttctgagtgctaag

SEQ ID NO: 65 - DNA, 18 bp, Artificial Sequence
  CPT1 Forward Primer
gctggaggtggctttggt

SEQ ID NO: 66 - DNA, 18 bp, Artificial Sequence
  CPT1 Reverse Primer
gcttggcggatgtggttc

SEQ ID NO: 67 - DNA, 23 bp, Artificial Sequence
  CPT2 Forward Primer
ggataaacagaataagcacacca

SEQ ID NO: 68 - DNA, 20 bp, Artificial Sequence
  CPT2 Reverse Primer
gaaggaacaaagcggatgag

SEQ ID NO: 69 - DNA, 19 bp, Artificial Sequence
  alpha-SMA Forward Primer
ccgaccgaatgcagaagga

SEQ ID NO: 70 - DNA, 21 bp, Artificial Sequence
  alpha-SMA Reverse Primer
acagagtatttgcgctccgaa

SEQ ID NO: 71 - DNA, 20 bp, Artificial Sequence
  Col1a1 Forward Primer
aaggtattgctggacagcgt

SEQ ID NO: 72 - DNA, 20 bp, Artificial Sequence
  Col1a1 Reverse Primer
tgtttgccaggttcaccaga

SEQ ID NO: 73 - DNA, 20 bp, Artificial Sequence
  MMP-3 Forward Primer
aacatctggcactccacacc

SEQ ID NO: 74 - DNA, 20 bp, Artificial Sequence
  MMP-3 Reverse Primer
gcagaagttctttggcctgc